European Patent Application EP 4 796 564 A1, published August 26, 2026. Title: 针对CCR8和CTLA4的双特异性抗体. Applicant: 普米斯生物技术（珠海）有限公司. Application WO. The sequence listing filed with the application follows.

SEQUENCE LISTING (161 sequences)

SEQ ID NO: 1 - protein, 120 aa, synthetic construct
EVQLVQSGAEVKKPGASVKVSCKASGYTFTSYYMHWVRQAPGQGLEWMGIINPGTGSTSHAQKFQGRVTMTRDTSTSTVYMELSSLRSEDTAVYYCARDGAFRHKYFDLWGRGTLVTVSS

SEQ ID NO: 2 - protein, 107 aa, synthetic construct
EIVLTQSPATLSLSPGERATLSCRASQSVSSYLAWYQQKPGQAPRLLIYDASNRATGIPARFSGSGSGTDFTLTISSLEPEDFAVYYCQQYSAWPLTFGGGTKVEIK

SEQ ID NO: 3 - protein, 118 aa, synthetic construct
EVQLVESGGGVVQPGRSLRLSCAASGFTFSSYTMHWVRQAPGKGLEWVTFISEDGNNKYYADSVKGRFTISRDNSKNTLYLQMNSLRAEDTAIYYCARTGWLGPFDYWGQGTLVTVSS

SEQ ID NO: 4 - protein, 108 aa, synthetic construct
DIVLTQSPGTLSLSPGERATLSCRASQSVGSSYLAWYQQKPGQAPRLLIYGAFSRATGIPDRFSGSGSGTDFTLTISRLEPEDFAVYYCQQYGSSPWTFGQGTKVEIK

SEQ ID NO: 5 - protein, 118 aa, synthetic construct
EVQLVESGGGVVQPGRSLRLSCAASGFTFSSYTMHWVRQAPGKGLEWVTFISEDGNNKYYADSVKGRFTISRDNSKNTLYLQMNSLRAEDTAIYYCARTGWLGPEDYWGQGTLVTVSS

SEQ ID NO: 6 - protein, 108 aa, synthetic construct; identical to SEQ ID NO: 4

SEQ ID NO: 7 - protein, 117 aa, synthetic construct
EVQLQESGGGLVQAGGSLTLSCAASGSIFSLNGMEWYRQFPGQQRELVAAITVGGSTIYADSVKGRFTISRDNAKNTVYLQMSSLKPEDTAVYYCHKFHFTLGQPYWGQGTQVTVSS

SEQ ID NO: 8 - protein, 116 aa, synthetic construct
EVQLQESGGGLVQAGGALRLSCAAPIDIFRISIMGWYRQAPGQQRELVARISKAGTTTYADSVKGRFTISRDNAKNTVILQMNSLKPEDTAVYYCNADRLRQHDLWGQGTQVTVSS

SEQ ID NO: 9 - protein, 119 aa, synthetic construct
EVQLQESGGGLVQPGGSLRLSCAASGIIFSIYHMGWYRQAPGKQRELVAVITSGGSTNYADSVKGRFTISRDNAKNTVYLQMNSLKPEDTAVYYCNSYHYGATRDYDAWGQGTQVTVSS

SEQ ID NO: 10 - protein, 119 aa, synthetic construct
EVQLQESGGGLVQPGGSLRLSCVASGSIFRPYVMGWYRQAPGKQRELVATNSKGGSTIYADAVKGRFTISSDNDENTVYLQMNSLKPEDTAVYYCNLKELGIYLRGDYWGQGTQVTVSS

SEQ ID NO: 11 - protein, 107 aa, synthetic construct [sequence omitted]

SEQ ID NO: 12 - protein, 329 aa, synthetic construct
ASTKGPSVFPLAPSSKSTSGGTAALGCLVKDYFPEPVTVSWNSGALTSGVHTFPAVLQSSGLYSLSSVVTVPSSSLGTQTYICNVNHKPSNTKVDKKVEPKSCDKTHTCPPCPAPELLGGPSVFLFPPKPKDTLMISRTPEVTCVVVDVSHEDPEVKFNWYVDGVEVHNAKTKPREEQYNSTYRVVSVLTVLHQDWLNGKEYKCKVSNKALPAPIEKTISKAKGQPREPQVYTLPPSRDELTKNQVSLTCLVKGFYPSDIAVEWESNGQPENNYKTTPPVLDSDGSFFLYSKLTVDKSRWQQGNVFSCSVMHEALHNHYTQKSLSLSPG

SEQ ID NO: 13 - protein, 329 aa, synthetic construct
ASTKGPSVFPLAPSSKSTSGGTAALGCLVKDYFPEPVTVSWNSGALTSGVHTFPAVLQSSGLYSLSSVVTVPSSSLGTQTYICNVNHKPSNTKVDKKVEPKSCDKTHTCPPCPAPELLGGPSVFLFPPKPKDTLMISRTPEVTCVVVDVSHEDPEVKFNWYVDGVEVHNAKTKPREEQYNSTYRVVSVLTVLHQDWLNGKEYKCKVSNKALPAPIEKTISKAKGQPREPQVYTLPPSRDELTKNQVSLTCLVKGFYPSDIAVEWESNGQPENNYKTTPPVLDSDGSFLLYSKLTVDKSRWQQGNVFSCSVMHEALHNHYTQKSLSLSPG

SEQ ID NO: 14 - protein, 329 aa, synthetic construct
ASTKGPSVFPLAPSSKSTSGGTAALGCLVKDYFPEPVTVSWNSGALTSGVHTFPAVLQSSGLYSLSSVVTVPSSSLGTQTYICNVNHKPSNTKVDKKVEPKSCDKTHTCPPCPAPELLGGPSVFLFPPKPKDTLMISRTPEVTCVVVDVSHEDPEVKFNWYVDGVEVHNAKTKPREEQYNSTYRVVSVLTVLHQDWLNGKEYKCKVSNKALPAPIEKTISKAKGQPREPQVYTLPPSRDELTKNQVSLTCLVKGFYPSDIAVEWESNGQPENNYKTTPPVLDSDGSFFLYSRLTVDKSRWQQGNVFSCSVMHEALHNHYTQKSLSLSPG

SEQ ID NO: 15 - protein, 226 aa, synthetic construct
DKTHTCPPCPAPELLGGPSVFLFPPKPKDTLMISRTPEVTCVVVDVSHEDPEVKFNWYVDGVEVHNAKTKPREEQYNSTYRVVSVLTVLHQDWLNGKEYKCKVSNKALPAPIEKTISKAKGQPREPQVYTLPPSRDELTKNQVSLTCLVKGFYPSDIAVEWESNGQPENNYKTTPPVLDSDGSFFLYSKLTVDKSRWQQGNVFSCSVMHEALHNHYTQKSLSLSPG

SEQ ID NO: 16 - protein, 226 aa, synthetic construct
DKTHTCPPCPAPELLGGPSVFLFPPKPKDTLMISRTPEVTCVVVDVSHEDPEVKFNWYVDGVEVHNAKTKPREEQYNSTYRVVSVLTVLHQDWLNGKEYKCKVSNKALPAPIEKTISKAKGQPREPQVYTLPPCRDELTKNQVSLWCLVKGFYPSDIAVEWESNGQPENNYKTTPPVLDSDGSFFLYSKLTVDKSRWQQGNVFSCSVMHEALHNHYTQKSLSLSPG

SEQ ID NO: 17 - protein, 329 aa, synthetic construct
ASTKGPSVFPLAPSSKSTSGGTAALGCLVKDYFPEPVTVSWNSGALTSGVHTFPAVLQSSGLYSLSSVVTVPSSSLGTQTYICNVNHKPSNTKVDKKVEPKSCDKTHTCPPCPAPELLGGPSVFLFPPKPKDTLMISRTPEVTCVVVDVSHEDPEVKFNWYVDGVEVHNAKTKPREEQYNSTYRVVSVLTVLHQDWLNGKEYKCKVSNKALPAPIEKTISKAKGQPREPQVCTLPPSRDELTKNQVSLSCAVKGFYPSDIAVEWESNGQPENNYKTTPPVLDSDGSFFLVSKLTVDKSRWQQGNVFSCSVMHEALHNRFTQKSLSLSPG

SEQ ID NO: 18 - protein, 449 aa, synthetic construct
EVQLVQSGAEVKKPGASVKVSCKASGYTFTSYYMHWVRQAPGQGLEWMGIINPGTGSTSHAQKFQGRVTMTRDTSTSTVYMELSSLRSEDTAVYYCARDGAFRHKYFDLWGRGTLVTVSSASTKGPSVFPLAPSSKSTSGGTAALGCLVKDYFPEPVTVSWNSGALTSGVHTFPAVLQSSGLYSLSSVVTVPSSSLGTQTYICNVNHKPSNTKVDKKVEPKSCDKTHTCPPCPAPELLGGPSVFLFPPKPKDTLMISRTPEVTCVVVDVSHEDPEVKFNWYVDGVEVHNAKTKPREEQYNSTYRVVSVLTVLHQDWLNGKEYKCKVSNKALPAPIEKTISKAKGQPREPQVYTLPPSRDELTKNQVSLTCLVKGFYPSDIAVEWESNGQPENNYKTTPPVLDSDGSFFLYSKLTVDKSRWQQGNVFSCSVMHEALHNHYTQKSLSLSPG

SEQ ID NO: 19 - protein, 214 aa, synthetic construct
EIVLTQSPATLSLSPGERATLSCRASQSVSSYLAWYQQKPGQAPRLLIYDASNRATGIPARFSGSGSGTDFTLTISSLEPEDFAVYYCQQYSAWPLTFGGGTKVEIKRTVAAPSVFIFPPSDEQLKSGTASVVCLLNNFYPREAKVQWKVDNALQSGNSQESVTEQDSKDSTYSLSSTLTLSKADYEKHKVYACEVTHQGLSSPVTKSFNRGEC

SEQ ID NO: 20 - protein, 447 aa, synthetic construct
EVQLVESGGGVVQPGRSLRLSCAASGFTFSSYTMHWVRQAPGKGLEWVTFISEDGNNKYYADSVKGRFTISRDNSKNTLYLQMNSLRAEDTAIYYCARTGWLGPFDYWGQGTLVTVSSASTKGPSVFPLAPSSKSTSGGTAALGCLVKDYFPEPVTVSWNSGALTSGVHTFPAVLQSSGLYSLSSVVTVPSSSLGTQTYICNVNHKPSNTKVDKKVEPKSCDKTHTCPPCPAPELLGGPSVFLFPPKPKDTLMISRTPEVTCVVVDVSHEDPEVKFNWYVDGVEVHNAKTKPREEQYNSTYRVVSVLTVLHQDWLNGKEYKCKVSNKALPAPIEKTISKAKGQPREPQVYTLPPSRDELTKNQVSLTCLVKGFYPSDIAVEWESNGQPENNYKTTPPVLDSDGSFFLYSKLTVDKSRWQQGNVFSCSVMHEALHNHYTQKSLSLSPG

SEQ ID NO: 21 - protein, 215 aa, synthetic construct
DIVLTQSPGTLSLSPGERATLSCRASQSVGSSYLAWYQQKPGQAPRLLIYGAFSRATGIPDRFSGSGSGTDFTLTISRLEPEDFAVYYCQQYGSSPWTFGQGTKVEIKRTVAAPSVFIFPPSDEQLKSGTASVVCLLNNFYPREAKVQWKVDNALQSGNSQESVTEQDSKDSTYSLSSTLTLSKADYEKHKVYACEVTHQGLSSPVTKSFNRGEC

SEQ ID NO: 22 - protein, 447 aa, synthetic construct
EVQLVESGGGVVQPGRSLRLSCAASGFTFSSYTMHWVRQAPGKGLEWVTFISEDGNNKYYADSVKGRFTISRDNSKNTLYLQMNSLRAEDTAIYYCARTGWLGPEDYWGQGTLVTVSSASTKGPSVFPLAPSSKSTSGGTAALGCLVKDYFPEPVTVSWNSGALTSGVHTFPAVLQSSGLYSLSSVVTVPSSSLGTQTYICNVNHKPSNTKVDKKVEPKSCDKTHTCPPCPAPELLGGPSVFLFPPKPKDTLMISRTPEVTCVVVDVSHEDPEVKFNWYVDGVEVHNAKTKPREEQYNSTYRVVSVLTVLHQDWLNGKEYKCKVSNKALPAPIEKTISKAKGQPREPQVYTLPPSRDELTKNQVSLTCLVKGFYPSDIAVEWESNGQPENNYKTTPPVLDSDGSFFLYSKLTVDKSRWQQGNVFSCSVMHEALHNHYTQKSLSLSPG

SEQ ID NO: 23 - protein, 215 aa, synthetic construct; identical to SEQ ID NO: 21

SEQ ID NO: 24 - protein, 343 aa, synthetic construct
EVQLQESGGGLVQAGGSLTLSCAASGSIFSLNGMEWYRQFPGQQRELVAAITVGGSTIYADSVKGRFTISRDNAKNTVYLQMSSLKPEDTAVYYCHKFHFTLGQPYWGQGTQVTVSSDKTHTCPPCPAPELLGGPSVFLFPPKPKDTLMISRTPEVTCVVVDVSHEDPEVKFNWYVDGVEVHNAKTKPREEQYNSTYRVVSVLTVLHQDWLNGKEYKCKVSNKALPAPIEKTISKAKGQPREPQVYTLPPSRDELTKNQVSLTCLVKGFYPSDIAVEWESNGQPENNYKTTPPVLDSDGSFFLYSKLTVDKSRWQQGNVFSCSVMHEALHNHYTQKSLSLSPG

SEQ ID NO: 25 - protein, 342 aa, synthetic construct
EVQLQESGGGLVQAGGALRLSCAAPIDIFRISIMGWYRQAPGQQRELVARISKAGTTTYADSVKGRFTISRDNAKNTVILQMNSLKPEDTAVYYCNADRLRQHDLWGQGTQVTVSSDKTHTCPPCPAPELLGGPSVFLFPPKPKDTLMISRTPEVTCVVVDVSHEDPEVKFNWYVDGVEVHNAKTKPREEQYNSTYRVVSVLTVLHQDWLNGKEYKCKVSNKALPAPIEKTISKAKGQPREPQVYTLPPSRDELTKNQVSLTCLVKGFYPSDIAVEWESNGQPENNYKTTPPVLDSDGSFFLYSKLTVDKSRWQQGNVFSCSVMHEALHNHYTQKSLSLSPG

SEQ ID NO: 26 - protein, 345 aa, synthetic construct
EVQLQESGGGLVQPGGSLRLSCAASGIIFSIYHMGWYRQAPGKQRELVAVITSGGSTNYADSVKGRFTISRDNAKNTVYLQMNSLKPEDTAVYYCNSYHYGATRDYDAWGQGTQVTVSSDKTHTCPPCPAPELLGGPSVFLFPPKPKDTLMISRTPEVTCVVVDVSHEDPEVKFNWYVDGVEVHNAKTKPREEQYNSTYRVVSVLTVLHQDWLNGKEYKCKVSNKALPAPIEKTISKAKGQPREPQVYTLPPSRDELTKNQVSLTCLVKGFYPSDIAVEWESNGQPENNYKTTPPVLDSDGSFFLYSKLTVDKSRWQQGNVFSCSVMHEALHNHYTQKSLSLSPG

SEQ ID NO: 27 - protein, 345 aa, synthetic construct
EVQLQESGGGLVQPGGSLRLSCVASGSIFRPYVMGWYRQAPGKQRELVATNSKGGSTIYADAVKGRFTISSDNDENTVYLQMNSLKPEDTAVYYCNLKELGIYLRGDYWGQGTQVTVSSDKTHTCPPCPAPELLGGPSVFLFPPKPKDTLMISRTPEVTCVVVDVSHEDPEVKFNWYVDGVEVHNAKTKPREEQYNSTYRVVSVLTVLHQDWLNGKEYKCKVSNKALPAPIEKTISKAKGQPREPQVYTLPPSRDELTKNQVSLTCLVKGFYPSDIAVEWESNGQPENNYKTTPPVLDSDGSFFLYSKLTVDKSRWQQGNVFSCSVMHEALHNHYTQKSLSLSPG

SEQ ID NO: 28 - protein, 447 aa, synthetic construct
EVQLVESGGGVVQPGRSLRLSCAASGFTFSSYTMHWVRQAPGKGLEWVTFISEDGNNKYYADSVKGRFTISRDNSKNTLYLQMNSLRAEDTAIYYCARTGWLGPFDYWGQGTLVTVSSASTKGPSVFPLAPSSKSTSGGTAALGCLVKDYFPEPVTVSWNSGALTSGVHTFPAVLQSSGLYSLSSVVTVPSSSLGTQTYICNVNHKPSNTKVDKKVEPKSCDKTHTCPPCPAPELLGGPSVFLFPPKPKDTLMISRTPEVTCVVVDVSHEDPEVKFNWYVDGVEVHNAKTKPREEQYNSTYRVVSVLTVLHQDWLNGKEYKCKVSNKALPAPIEKTISKAKGQPREPQVYTLPPSRDELTKNQVSLTCLVKGFYPSDIAVEWESNGQPENNYKTTPPVLDSDGSFLLYSKLTVDKSRWQQGNVFSCSVMHEALHNHYTQKSLSLSPG

SEQ ID NO: 29 - protein, 215 aa, synthetic construct; identical to SEQ ID NO: 21

SEQ ID NO: 30 - protein, 449 aa, synthetic construct
EVQLVQSGAEVKKPGASVKVSCKASGYTFTSYYMHWVRQAPGQGLEWMGIINPGTGSTSHAQKFQGRVTMTRDTSTSTVYMELSSLRSEDTAVYYCARDGAFRHKYFDLWGRGTLVTVSSASTKGPSVFPLAPSSKSTSGGTAALGCLVKDYFPEPVTVSWNSGALTSGVHTFPAVLQSSGLYSLSSVVTVPSSSLGTQTYICNVNHKPSNTKVDKKVEPKSCDKTHTCPPCPAPELLGGPSVFLFPPKPKDTLMISRTPEVTCVVVDVSHEDPEVKFNWYVDGVEVHNAKTKPREEQYNSTYRVVSVLTVLHQDWLNGKEYKCKVSNKALPAPIEKTISKAKGQPREPQVYTLPPSRDELTKNQVSLTCLVKGFYPSDIAVEWESNGQPENNYKTTPPVLDSDGSFFLYSRLTVDKSRWQQGNVFSCSVMHEALHNHYTQKSLSLSPG

SEQ ID NO: 31 - protein, 214 aa, synthetic construct; identical to SEQ ID NO: 19

SEQ ID NO: 32 - protein, 447 aa, synthetic construct
EVQLVESGGGVVQPGRSLRLSCAASGFTFSSYTMHWVRQAPGKGLEWVTFISEDGNNKYYADSVKGRFTISRDNSKNTLYLQMNSLRAEDTAIYYCARTGWLGPEDYWGQGTLVTVSSASTKGPSVFPLAPSSKSTSGGTAALGCLVKDYFPEPVTVSWNSGALTSGVHTFPAVLQSSGLYSLSSVVTVPSSSLGTQTYICNVNHKPSNTKVDKKVEPKSCDKTHTCPPCPAPELLGGPSVFLFPPKPKDTLMISRTPEVTCVVVDVSHEDPEVKFNWYVDGVEVHNAKTKPREEQYNSTYRVVSVLTVLHQDWLNGKEYKCKVSNKALPAPIEKTISKAKGQPREPQVYTLPPSRDELTKNQVSLTCLVKGFYPSDIAVEWESNGQPENNYKTTPPVLDSDGSFLLYSKLTVDKSRWQQGNVFSCSVMHEALHNHYTQKSLSLSPG

SEQ ID NO: 33 - protein, 215 aa, synthetic construct; identical to SEQ ID NO: 21

SEQ ID NO: 34 - protein, 449 aa, synthetic construct; identical to SEQ ID NO: 30

SEQ ID NO: 35 - protein, 214 aa, synthetic construct; identical to SEQ ID NO: 19

SEQ ID NO: 36 - protein, 343 aa, synthetic construct
EVQLQESGGGLVQAGGSLTLSCAASGSIFSLNGMEWYRQFPGQQRELVAAITVGGSTIYADSVKGRFTISRDNAKNTVYLQMSSLKPEDTAVYYCHKFHFTLGQPYWGQGTQVTVSSDKTHTCPPCPAPELLGGPSVFLFPPKPKDTLMISRTPEVTCVVVDVSHEDPEVKFNWYVDGVEVHNAKTKPREEQYNSTYRVVSVLTVLHQDWLNGKEYKCKVSNKALPAPIEKTISKAKGQPREPQVYTLPPCRDELTKNQVSLWCLVKGFYPSDIAVEWESNGQPENNYKTTPPVLDSDGSFFLYSKLTVDKSRWQQGNVFSCSVMHEALHNHYTQKSLSLSPG

SEQ ID NO: 37 - protein, 449 aa, synthetic construct
EVQLVQSGAEVKKPGASVKVSCKASGYTFTSYYMHWVRQAPGQGLEWMGIINPGTGSTSHAQKFQGRVTMTRDTSTSTVYMELSSLRSEDTAVYYCARDGAFRHKYFDLWGRGTLVTVSSASTKGPSVFPLAPSSKSTSGGTAALGCLVKDYFPEPVTVSWNSGALTSGVHTFPAVLQSSGLYSLSSVVTVPSSSLGTQTYICNVNHKPSNTKVDKKVEPKSCDKTHTCPPCPAPELLGGPSVFLFPPKPKDTLMISRTPEVTCVVVDVSHEDPEVKFNWYVDGVEVHNAKTKPREEQYNSTYRVVSVLTVLHQDWLNGKEYKCKVSNKALPAPIEKTISKAKGQPREPQVCTLPPSRDELTKNQVSLSCAVKGFYPSDIAVEWESNGQPENNYKTTPPVLDSDGSFFLVSKLTVDKSRWQQGNVFSCSVMHEALHNRFTQKSLSLSPG

SEQ ID NO: 38 - protein, 214 aa, synthetic construct; identical to SEQ ID NO: 19

SEQ ID NO: 39 - protein, 342 aa, synthetic construct
EVQLQESGGGLVQAGGALRLSCAAPIDIFRISIMGWYRQAPGQQRELVARISKAGTTTYADSVKGRFTISRDNAKNTVILQMNSLKPEDTAVYYCNADRLRQHDLWGQGTQVTVSSDKTHTCPPCPAPELLGGPSVFLFPPKPKDTLMISRTPEVTCVVVDVSHEDPEVKFNWYVDGVEVHNAKTKPREEQYNSTYRVVSVLTVLHQDWLNGKEYKCKVSNKALPAPIEKTISKAKGQPREPQVYTLPPCRDELTKNQVSLWCLVKGFYPSDIAVEWESNGQPENNYKTTPPVLDSDGSFFLYSKLTVDKSRWQQGNVFSCSVMHEALHNHYTQKSLSLSPG

SEQ ID NO: 40 - protein, 449 aa, synthetic construct; identical to SEQ ID NO: 37

SEQ ID NO: 41 - protein, 214 aa, synthetic construct; identical to SEQ ID NO: 19

SEQ ID NO: 42 - protein, 345 aa, synthetic construct
EVQLQESGGGLVQPGGSLRLSCAASGIIFSIYHMGWYRQAPGKQRELVAVITSGGSTNYADSVKGRFTISRDNAKNTVYLQMNSLKPEDTAVYYCNSYHYGATRDYDAWGQGTQVTVSSDKTHTCPPCPAPELLGGPSVFLFPPKPKDTLMISRTPEVTCVVVDVSHEDPEVKFNWYVDGVEVHNAKTKPREEQYNSTYRVVSVLTVLHQDWLNGKEYKCKVSNKALPAPIEKTISKAKGQPREPQVYTLPPCRDELTKNQVSLWCLVKGFYPSDIAVEWESNGQPENNYKTTPPVLDSDGSFFLYSKLTVDKSRWQQGNVFSCSVMHEALHNHYTQKSLSLSPG

SEQ ID NO: 43 - protein, 449 aa, synthetic construct; identical to SEQ ID NO: 37

SEQ ID NO: 44 - protein, 214 aa, synthetic construct; identical to SEQ ID NO: 19

SEQ ID NO: 45 - protein, 345 aa, synthetic construct
EVQLQESGGGLVQPGGSLRLSCVASGSIFRPYVMGWYRQAPGKQRELVATNSKGGSTIYADAVKGRFTISSDNDENTVYLQMNSLKPEDTAVYYCNLKELGIYLRGDYWGQGTQVTVSSDKTHTCPPCPAPELLGGPSVFLFPPKPKDTLMISRTPEVTCVVVDVSHEDPEVKFNWYVDGVEVHNAKTKPREEQYNSTYRVVSVLTVLHQDWLNGKEYKCKVSNKALPAPIEKTISKAKGQPREPQVYTLPPCRDELTKNQVSLWCLVKGFYPSDIAVEWESNGQPENNYKTTPPVLDSDGSFFLYSKLTVDKSRWQQGNVFSCSVMHEALHNHYTQKSLSLSPG

SEQ ID NO: 46 - protein, 449 aa, synthetic construct; identical to SEQ ID NO: 37

SEQ ID NO: 47 - protein, 214 aa, synthetic construct; identical to SEQ ID NO: 19

SEQ ID NO: 48 - protein, 8 aa, synthetic construct
GFTFSSYT

SEQ ID NO: 49 - protein, 8 aa, synthetic construct
ISEDGNNK

SEQ ID NO: 50 - protein, 11 aa, synthetic construct
ARTGWLGPFDY

SEQ ID NO: 51 - protein, 7 aa, synthetic construct
QSVGSSY

SEQ ID NO: 52 - skipped

SEQ ID NO: 53 - protein, 9 aa, synthetic construct
QQYGSSPWT

SEQ ID NO: 54 - protein, 8 aa, synthetic construct
GFTFSSYT

SEQ ID NO: 55 - protein, 8 aa, synthetic construct
ISEDGNNK

SEQ ID NO: 56 - protein, 11 aa, synthetic construct
ARTGWLGPEDY

SEQ ID NO: 57 - protein, 7 aa, synthetic construct
QSVGSSY

SEQ ID NO: 58 - skipped

SEQ ID NO: 59 - protein, 9 aa, synthetic construct
QQYGSSPWT

SEQ ID NO: 60 - protein, 8 aa, synthetic construct
GSIFSLNG

SEQ ID NO: 61 - protein, 7 aa, synthetic construct
ITVGGST

SEQ ID NO: 62 - protein, 11 aa, synthetic construct
HKFHFTLGQPY

SEQ ID NO: 63 - protein, 8 aa, synthetic construct
IDIFRISI

SEQ ID NO: 64 - protein, 7 aa, synthetic construct
ISKAGTT

SEQ ID NO: 65 - protein, 10 aa, synthetic construct
NADRLRQHDL

SEQ ID NO: 66 - protein, 8 aa, synthetic construct
GIIFSIYH

SEQ ID NO: 67 - protein, 7 aa, synthetic construct
ITSGGST

SEQ ID NO: 68 - protein, 13 aa, synthetic construct
NSYHYGATRDYDA

SEQ ID NO: 69 - protein, 8 aa, synthetic construct
GSIFRPYV

SEQ ID NO: 70 - protein, 7 aa, synthetic construct
NSKGGST

SEQ ID NO: 71 - protein, 13 aa, synthetic construct
NLKELGIYLRGDY

SEQ ID NO: 72 - protein, 8 aa, synthetic construct
GYTFTSYY

SEQ ID NO: 73 - protein, 8 aa, synthetic construct
INPGTGST

SEQ ID NO: 74 - protein, 13 aa, synthetic construct
ARDGAFRHKYFDL

SEQ ID NO: 75 - protein, 6 aa, synthetic construct
QSVSSY

SEQ ID NO: 76 - skipped

SEQ ID NO: 77 - protein, 9 aa, synthetic construct
QQYSAWPLT

SEQ ID NO: 78 - protein, 120 aa, synthetic construct
EVQLVQSGAEVKKPGASVKVSCKASGYTFTSYYMHWVRQAPGQGLEWMGIINPMTGSASHAQKFQGRVTMTRDTSTSTVYMELSSLRSEDTAVYYCVRDAAARHKYFAFWGRGTLVTVSS

SEQ ID NO: 79 - protein, 329 aa, synthetic construct
ASTKGPSVFPLAPSSKSTSGGTAALGCQVEDYFPEPVTVSWNSGALTSGVHTFPAVLQSSGLYELSSVVTVPSSSLGTQTYICNVNHKPSNTKVDKKVEPKSCDKTHTCPPCPAPELLGGPSVFLFPPKPKDTLMISRTPEVTCVVVDVSHEDPEVKFNWYVDGVEVHNAKTKPREEQYNSTYRVVSVLTVLHQDWLNGKEYKCKVSNKALPAPIEKTISKAKGQPREPQVYTLPPCRDELTKNQVSLWCLVKGFYPSDIAVEWESNGQPENNYKTTPPVLDSDGSFFLYSKLTVDKSRWQQGNVFSCSVMHEALHNHYTQKSLSLSPG

SEQ ID NO: 80 - protein, 329 aa, synthetic construct
ASTKGPSVFPRAPSSKSTSGGTAALGCLVRDYFPEPVTVSWNSGALTSGVHTFPAVLQSSGLYSLSSVVTVPSSSLGTQTYICNVNHKPSNTKVDKKVEPKSCDKTHTCPPCPAPELLGGPSVFLFPPKPKDTLMISRTPEVTCVVVDVSHEDPEVKFNWYVDGVEVHNAKTKPREEQYNSTYRVVSVLTVLHQDWLNGKEYKCKVSNKALPAPIEKTISKAKGQPREPQVCTLPPSRDELTKNQVSLSCAVKGFYPSDIAVEWESNGQPENNYKTTPPVLDSDGSFFLVSKLTVDKSRWQQGNVFSCSVMHEALHNHYTQKSLSLSPG

SEQ ID NO: 81 - protein, 107 aa, synthetic construct
RTVAAPSVFIFPPSDEQLKSGRASVVCLLNNFYPREAKVQWKVDNALQSGNSQESVTEQDSKDSTYSLSSRLQLSKADYEKHKVYACEVTHQGLSSPVTKSFNRGEC

SEQ ID NO: 82 - protein, 107 aa, synthetic construct
RTVAAPSVFIFPPSDEELKSGTASVQCLLNNFYPREAKVQWKVDNALQSGNSQESVTEQDSKDSTYSLSSELTLSKADYEKHKVYACEVTHQGLSSPVTKSFNRGEC

SEQ ID NO: 83 - protein, 449 aa, synthetic construct
EVQLVQSGAEVKKPGASVKVSCKASGYTFTSYYMHWVRQAPGQGLEWMGIINPMTGSASHAQKFQGRVTMTRDTSTSTVYMELSSLRSEDTAVYYCVRDAAARHKYFAFWGRGTLVTVSSASTKGPSVFPLAPSSKSTSGGTAALGCLVKDYFPEPVTVSWNSGALTSGVHTFPAVLQSSGLYSLSSVVTVPSSSLGTQTYICNVNHKPSNTKVDKKVEPKSCDKTHTCPPCPAPELLGGPSVFLFPPKPKDTLMISRTPEVTCVVVDVSHEDPEVKFNWYVDGVEVHNAKTKPREEQYNSTYRVVSVLTVLHQDWLNGKEYKCKVSNKALPAPIEKTISKAKGQPREPQVYTLPPSRDELTKNQVSLTCLVKGFYPSDIAVEWESNGQPENNYKTTPPVLDSDGSFFLYSKLTVDKSRWQQGNVFSCSVMHEALHNHYTQKSLSLSPG

SEQ ID NO: 84 - protein, 214 aa, synthetic construct; identical to SEQ ID NO: 19

SEQ ID NO: 85 - protein, 447 aa, synthetic construct; identical to SEQ ID NO: 28

SEQ ID NO: 86 - protein, 215 aa, synthetic construct; identical to SEQ ID NO: 21

SEQ ID NO: 87 - protein, 449 aa, synthetic construct
EVQLVQSGAEVKKPGASVKVSCKASGYTFTSYYMHWVRQAPGQGLEWMGIINPMTGSASHAQKFQGRVTMTRDTSTSTVYMELSSLRSEDTAVYYCVRDAAARHKYFAFWGRGTLVTVSSASTKGPSVFPLAPSSKSTSGGTAALGCLVKDYFPEPVTVSWNSGALTSGVHTFPAVLQSSGLYSLSSVVTVPSSSLGTQTYICNVNHKPSNTKVDKKVEPKSCDKTHTCPPCPAPELLGGPSVFLFPPKPKDTLMISRTPEVTCVVVDVSHEDPEVKFNWYVDGVEVHNAKTKPREEQYNSTYRVVSVLTVLHQDWLNGKEYKCKVSNKALPAPIEKTISKAKGQPREPQVYTLPPSRDELTKNQVSLTCLVKGFYPSDIAVEWESNGQPENNYKTTPPVLDSDGSFFLYSRLTVDKSRWQQGNVFSCSVMHEALHNHYTQKSLSLSPG

SEQ ID NO: 88 - protein, 214 aa, synthetic construct; identical to SEQ ID NO: 19

SEQ ID NO: 89 - protein, 447 aa, synthetic construct; identical to SEQ ID NO: 32

SEQ ID NO: 90 - protein, 215 aa, synthetic construct; identical to SEQ ID NO: 21

SEQ ID NO: 91 - protein, 449 aa, synthetic construct; identical to SEQ ID NO: 87

SEQ ID NO: 92 - protein, 214 aa, synthetic construct; identical to SEQ ID NO: 19

SEQ ID NO: 93 - protein, 449 aa, synthetic construct
EVQLVQSGAEVKKPGASVKVSCKASGYTFTSYYMHWVRQAPGQGLEWMGIINPGTGSTSHAQKFQGRVTMTRDTSTSTVYMELSSLRSEDTAVYYCARDGAFRHKYFDLWGRGTLVTVSSASTKGPSVFPLAPSSKSTSGGTAALGCQVEDYFPEPVTVSWNSGALTSGVHTFPAVLQSSGLYELSSVVTVPSSSLGTQTYICNVNHKPSNTKVDKKVEPKSCDKTHTCPPCPAPELLGGPSVFLFPPKPKDTLMISRTPEVTCVVVDVSHEDPEVKFNWYVDGVEVHNAKTKPREEQYNSTYRVVSVLTVLHQDWLNGKEYKCKVSNKALPAPIEKTISKAKGQPREPQVYTLPPCRDELTKNQVSLWCLVKGFYPSDIAVEWESNGQPENNYKTTPPVLDSDGSFFLYSKLTVDKSRWQQGNVFSCSVMHEALHNHYTQKSLSLSPG

SEQ ID NO: 94 - protein, 214 aa, synthetic construct
EIVLTQSPATLSLSPGERATLSCRASQSVSSYLAWYQQKPGQAPRLLIYDASNRATGIPARFSGSGSGTDFTLTISSLEPEDFAVYYCQQYSAWPLTFGGGTKVEIKRTVAAPSVFIFPPSDEQLKSGRASVVCLLNNFYPREAKVQWKVDNALQSGNSQESVTEQDSKDSTYSLSSRLQLSKADYEKHKVYACEVTHQGLSSPVTKSFNRGEC

SEQ ID NO: 95 - protein, 447 aa, synthetic construct
EVQLVESGGGVVQPGRSLRLSCAASGFTFSSYTMHWVRQAPGKGLEWVTFISEDGNNKYYADSVKGRFTISRDNSKNTLYLQMNSLRAEDTAIYYCARTGWLGPFDYWGQGTLVTVSSASTKGPSVFPRAPSSKSTSGGTAALGCLVRDYFPEPVTVSWNSGALTSGVHTFPAVLQSSGLYSLSSVVTVPSSSLGTQTYICNVNHKPSNTKVDKKVEPKSCDKTHTCPPCPAPELLGGPSVFLFPPKPKDTLMISRTPEVTCVVVDVSHEDPEVKFNWYVDGVEVHNAKTKPREEQYNSTYRVVSVLTVLHQDWLNGKEYKCKVSNKALPAPIEKTISKAKGQPREPQVCTLPPSRDELTKNQVSLSCAVKGFYPSDIAVEWESNGQPENNYKTTPPVLDSDGSFFLVSKLTVDKSRWQQGNVFSCSVMHEALHNHYTQKSLSLSPG

SEQ ID NO: 96 - protein, 215 aa, synthetic construct
DIVLTQSPGTLSLSPGERATLSCRASQSVGSSYLAWYQQKPGQAPRLLIYGAFSRATGIPDRFSGSGSGTDFTLTISRLEPEDFAVYYCQQYGSSPWTFGQGTKVEIKRTVAAPSVFIFPPSDEELKSGTASVQCLLNNFYPREAKVQWKVDNALQSGNSQESVTEQDSKDSTYSLSSELTLSKADYEKHKVYACEVTHQGLSSPVTKSFNRGEC

SEQ ID NO: 97 - protein, 449 aa, synthetic construct
EVQLVQSGAEVKKPGASVKVSCKASGYTFTSYYMHWVRQAPGQGLEWMGIINPMTGSASHAQKFQGRVTMTRDTSTSTVYMELSSLRSEDTAVYYCVRDAAARHKYFAFWGRGTLVTVSSASTKGPSVFPLAPSSKSTSGGTAALGCQVEDYFPEPVTVSWNSGALTSGVHTFPAVLQSSGLYELSSVVTVPSSSLGTQTYICNVNHKPSNTKVDKKVEPKSCDKTHTCPPCPAPELLGGPSVFLFPPKPKDTLMISRTPEVTCVVVDVSHEDPEVKFNWYVDGVEVHNAKTKPREEQYNSTYRVVSVLTVLHQDWLNGKEYKCKVSNKALPAPIEKTISKAKGQPREPQVYTLPPCRDELTKNQVSLWCLVKGFYPSDIAVEWESNGQPENNYKTTPPVLDSDGSFFLYSKLTVDKSRWQQGNVFSCSVMHEALHNHYTQKSLSLSPG

SEQ ID NO: 98 - protein, 214 aa, synthetic construct; identical to SEQ ID NO: 94

SEQ ID NO: 99 - protein, 447 aa, synthetic construct; identical to SEQ ID NO: 95

SEQ ID NO: 100 - protein, 215 aa, synthetic construct; identical to SEQ ID NO: 96

SEQ ID NO: 101 - protein, 449 aa, synthetic construct; identical to SEQ ID NO: 93

SEQ ID NO: 102 - protein, 214 aa, synthetic construct; identical to SEQ ID NO: 94

SEQ ID NO: 103 - protein, 447 aa, synthetic construct
EVQLVESGGGVVQPGRSLRLSCAASGFTFSSYTMHWVRQAPGKGLEWVTFISEDGNNKYYADSVKGRFTISRDNSKNTLYLQMNSLRAEDTAIYYCARTGWLGPEDYWGQGTLVTVSSASTKGPSVFPRAPSSKSTSGGTAALGCLVRDYFPEPVTVSWNSGALTSGVHTFPAVLQSSGLYSLSSVVTVPSSSLGTQTYICNVNHKPSNTKVDKKVEPKSCDKTHTCPPCPAPELLGGPSVFLFPPKPKDTLMISRTPEVTCVVVDVSHEDPEVKFNWYVDGVEVHNAKTKPREEQYNSTYRVVSVLTVLHQDWLNGKEYKCKVSNKALPAPIEKTISKAKGQPREPQVCTLPPSRDELTKNQVSLSCAVKGFYPSDIAVEWESNGQPENNYKTTPPVLDSDGSFFLVSKLTVDKSRWQQGNVFSCSVMHEALHNHYTQKSLSLSPG

SEQ ID NO: 104 - protein, 215 aa, synthetic construct; identical to SEQ ID NO: 96

SEQ ID NO: 105 - protein, 449 aa, synthetic construct; identical to SEQ ID NO: 97

SEQ ID NO: 106 - protein, 214 aa, synthetic construct; identical to SEQ ID NO: 94

SEQ ID NO: 107 - protein, 447 aa, synthetic construct; identical to SEQ ID NO: 103

SEQ ID NO: 108 - protein, 215 aa, synthetic construct; identical to SEQ ID NO: 96

SEQ ID NO: 109 - protein, 447 aa, synthetic construct
EVQLVESGGGVVQPGRSLRLSCAASGFTFSSYTMHWVRQAPGKGLEWVTFISEDGNNKYYADSVKGRFTISRDNSKNTLYLQMNSLRAEDTAIYYCARTGWLGPFDYWGQGTLVTVSSASTKGPSVFPLAPSSKSTSGGTAALGCQVEDYFPEPVTVSWNSGALTSGVHTFPAVLQSSGLYELSSVVTVPSSSLGTQTYICNVNHKPSNTKVDKKVEPKSCDKTHTCPPCPAPELLGGPSVFLFPPKPKDTLMISRTPEVTCVVVDVSHEDPEVKFNWYVDGVEVHNAKTKPREEQYNSTYRVVSVLTVLHQDWLNGKEYKCKVSNKALPAPIEKTISKAKGQPREPQVYTLPPCRDELTKNQVSLWCLVKGFYPSDIAVEWESNGQPENNYKTTPPVLDSDGSFFLYSKLTVDKSRWQQGNVFSCSVMHEALHNHYTQKSLSLSPG

SEQ ID NO: 110 - protein, 215 aa, synthetic construct
DIVLTQSPGTLSLSPGERATLSCRASQSVGSSYLAWYQQKPGQAPRLLIYGAFSRATGIPDRFSGSGSGTDFTLTISRLEPEDFAVYYCQQYGSSPWTFGQGTKVEIKRTVAAPSVFIFPPSDEQLKSGRASVVCLLNNFYPREAKVQWKVDNALQSGNSQESVTEQDSKDSTYSLSSRLQLSKADYEKHKVYACEVTHQGLSSPVTKSFNRGEC

SEQ ID NO: 111 - protein, 449 aa, synthetic construct
EVQLVQSGAEVKKPGASVKVSCKASGYTFTSYYMHWVRQAPGQGLEWMGIINPGTGSTSHAQKFQGRVTMTRDTSTSTVYMELSSLRSEDTAVYYCARDGAFRHKYFDLWGRGTLVTVSSASTKGPSVFPRAPSSKSTSGGTAALGCLVRDYFPEPVTVSWNSGALTSGVHTFPAVLQSSGLYSLSSVVTVPSSSLGTQTYICNVNHKPSNTKVDKKVEPKSCDKTHTCPPCPAPELLGGPSVFLFPPKPKDTLMISRTPEVTCVVVDVSHEDPEVKFNWYVDGVEVHNAKTKPREEQYNSTYRVVSVLTVLHQDWLNGKEYKCKVSNKALPAPIEKTISKAKGQPREPQVCTLPPSRDELTKNQVSLSCAVKGFYPSDIAVEWESNGQPENNYKTTPPVLDSDGSFFLVSKLTVDKSRWQQGNVFSCSVMHEALHNHYTQKSLSLSPG

SEQ ID NO: 112 - protein, 214 aa, synthetic construct
EIVLTQSPATLSLSPGERATLSCRASQSVSSYLAWYQQKPGQAPRLLIYDASNRATGIPARFSGSGSGTDFTLTISSLEPEDFAVYYCQQYSAWPLTFGGGTKVEIKRTVAAPSVFIFPPSDEELKSGTASVQCLLNNFYPREAKVQWKVDNALQSGNSQESVTEQDSKDSTYSLSSELTLSKADYEKHKVYACEVTHQGLSSPVTKSFNRGEC

SEQ ID NO: 113 - protein, 447 aa, synthetic construct; identical to SEQ ID NO: 109

SEQ ID NO: 114 - protein, 215 aa, synthetic construct; identical to SEQ ID NO: 110

SEQ ID NO: 115 - protein, 449 aa, synthetic construct
EVQLVQSGAEVKKPGASVKVSCKASGYTFTSYYMHWVRQAPGQGLEWMGIINPMTGSASHAQKFQGRVTMTRDTSTSTVYMELSSLRSEDTAVYYCVRDAAARHKYFAFWGRGTLVTVSSASTKGPSVFPRAPSSKSTSGGTAALGCLVRDYFPEPVTVSWNSGALTSGVHTFPAVLQSSGLYSLSSVVTVPSSSLGTQTYICNVNHKPSNTKVDKKVEPKSCDKTHTCPPCPAPELLGGPSVFLFPPKPKDTLMISRTPEVTCVVVDVSHEDPEVKFNWYVDGVEVHNAKTKPREEQYNSTYRVVSVLTVLHQDWLNGKEYKCKVSNKALPAPIEKTISKAKGQPREPQVCTLPPSRDELTKNQVSLSCAVKGFYPSDIAVEWESNGQPENNYKTTPPVLDSDGSFFLVSKLTVDKSRWQQGNVFSCSVMHEALHNHYTQKSLSLSPG

SEQ ID NO: 116 - protein, 214 aa, synthetic construct; identical to SEQ ID NO: 112

SEQ ID NO: 117 - protein, 447 aa, synthetic construct
EVQLVESGGGVVQPGRSLRLSCAASGFTFSSYTMHWVRQAPGKGLEWVTFISEDGNNKYYADSVKGRFTISRDNSKNTLYLQMNSLRAEDTAIYYCARTGWLGPEDYWGQGTLVTVSSASTKGPSVFPLAPSSKSTSGGTAALGCQVEDYFPEPVTVSWNSGALTSGVHTFPAVLQSSGLYELSSVVTVPSSSLGTQTYICNVNHKPSNTKVDKKVEPKSCDKTHTCPPCPAPELLGGPSVFLFPPKPKDTLMISRTPEVTCVVVDVSHEDPEVKFNWYVDGVEVHNAKTKPREEQYNSTYRVVSVLTVLHQDWLNGKEYKCKVSNKALPAPIEKTISKAKGQPREPQVYTLPPCRDELTKNQVSLWCLVKGFYPSDIAVEWESNGQPENNYKTTPPVLDSDGSFFLYSKLTVDKSRWQQGNVFSCSVMHEALHNHYTQKSLSLSPG

SEQ ID NO: 118 - protein, 215 aa, synthetic construct; identical to SEQ ID NO: 110

SEQ ID NO: 119 - protein, 449 aa, synthetic construct; identical to SEQ ID NO: 111

SEQ ID NO: 120 - protein, 214 aa, synthetic construct; identical to SEQ ID NO: 112

SEQ ID NO: 121 - protein, 447 aa, synthetic construct; identical to SEQ ID NO: 117

SEQ ID NO: 122 - protein, 215 aa, synthetic construct; identical to SEQ ID NO: 110

SEQ ID NO: 123 - protein, 449 aa, synthetic construct; identical to SEQ ID NO: 115

SEQ ID NO: 124 - protein, 214 aa, synthetic construct; identical to SEQ ID NO: 112

SEQ ID NO: 125 - protein, 343 aa, synthetic construct; identical to SEQ ID NO: 36

SEQ ID NO: 126 - protein, 449 aa, synthetic construct
EVQLVQSGAEVKKPGASVKVSCKASGYTFTSYYMHWVRQAPGQGLEWMGIINPMTGSASHAQKFQGRVTMTRDTSTSTVYMELSSLRSEDTAVYYCVRDAAARHKYFAFWGRGTLVTVSSASTKGPSVFPLAPSSKSTSGGTAALGCLVKDYFPEPVTVSWNSGALTSGVHTFPAVLQSSGLYSLSSVVTVPSSSLGTQTYICNVNHKPSNTKVDKKVEPKSCDKTHTCPPCPAPELLGGPSVFLFPPKPKDTLMISRTPEVTCVVVDVSHEDPEVKFNWYVDGVEVHNAKTKPREEQYNSTYRVVSVLTVLHQDWLNGKEYKCKVSNKALPAPIEKTISKAKGQPREPQVCTLPPSRDELTKNQVSLSCAVKGFYPSDIAVEWESNGQPENNYKTTPPVLDSDGSFFLVSKLTVDKSRWQQGNVFSCSVMHEALHNRFTQKSLSLSPG

SEQ ID NO: 127 - protein, 214 aa, synthetic construct; identical to SEQ ID NO: 19

SEQ ID NO: 128 - protein, 342 aa, synthetic construct; identical to SEQ ID NO: 39

SEQ ID NO: 129 - protein, 449 aa, synthetic construct; identical to SEQ ID NO: 126

SEQ ID NO: 130 - protein, 214 aa, synthetic construct; identical to SEQ ID NO: 19

SEQ ID NO: 131 - protein, 345 aa, synthetic construct; identical to SEQ ID NO: 42

SEQ ID NO: 132 - protein, 449 aa, synthetic construct; identical to SEQ ID NO: 126

SEQ ID NO: 133 - protein, 214 aa, synthetic construct; identical to SEQ ID NO: 19

SEQ ID NO: 134 - protein, 345 aa, synthetic construct; identical to SEQ ID NO: 45

SEQ ID NO: 135 - protein, 449 aa, synthetic construct; identical to SEQ ID NO: 126

SEQ ID NO: 136 - protein, 214 aa, synthetic construct; identical to SEQ ID NO: 19

SEQ ID NO: 137 - protein, 8 aa, synthetic construct
GYTFTSYY

SEQ ID NO: 138 - protein, 8 aa, synthetic construct
INPMTGSA

SEQ ID NO: 139 - protein, 13 aa, synthetic construct
VRDAAARHKYFAF

SEQ ID NO: 140 - protein, 329 aa, synthetic construct
AKTTAPSVYPLAPVCGDTTGSSVTLGCLVKGYFPEPVTLTWNSGSLSSGVHTFPAVLQSDLYTLSSSVTVTSSTWPSQSITCNVAHPASSTKVDKKIEPRGPTIKPCPPCKCPAPNLLGGPSVFIFPPKIKDVLMISLSPIVTCVVVDVSEDDPDVQISWFVNNVEVHTAQTQTHREDYNSTLRVVSALPIQHQDWMSGKEFKCKVNNKDLPAPIERTISKPKGSVRAPQVYVLPPPEEEMTKKQVTLTCMVTDFMPEDIYVEWTNNGKTELNYKNTEPVLDSDGSYLMYSKLTVEKKNWVERNSYSCSVVHEGLHNHHTTKSFSRTPG

SEQ ID NO: 141 - protein, 329 aa, synthetic construct
AKTTAPSVYPLAPVCGDTTGSSVTLGCLVKGYFPEPVTLTWNSGSLSSGVHTFPAVLQSDLYTLSSSVTVTSSTWPSQSITCNVAHPASSTKVDKKIEPRGPTIKPCPPCKCPAPNLLGGPSVFIFPPKIKDVLMISLSPIVTCVVVDVSEDDPDVQISWFVNNVEVHTAQTQTHREDYNSTLRVVSALPIQHQDWMSGKEFKCKVNNKDLPAPIERTISKPKGSVRAPQVYVLPPPEEEMTKKQVTLTCMVKDFMPEDIYVEWTNNGKTELNYKNTEPVLDSDGSYFMYSRLRVEKKNWVERNSYSCSVVHEGLHNRFTTKSFSRTPG

SEQ ID NO: 142 - protein, 329 aa, synthetic construct
AKTTAPSVYPLAPVCGDTTGSSVTLGCLVKGYFPEPVTLTWNSGSLSSGVHTFPAVLQSDLYTLSSSVTVTSSTWPSQSITCNVAHPASSTKVDKKIEPRGPTIKPCPPCKCPAPNLLGGPSVFIFPPKIKDVLMISLSPIVTCVVVDVSEDDPDVQISWFVNNVEVHTAQTQTHREDYNSTLRVVSALPIQHQDWMSGKEFKCKVNNKDLPAPIERTISKPKGSVRAPQVYVLPPPEEEMTKKQVTLTCMVTDFMPEDIYVEWTNNGKTELNYKNTEPVLDSDGSYFMYSKLRVEKKNWVERNSYSCSVVHEGLHNHHTTKSFSRTPG

SEQ ID NO: 143 - protein, 107 aa, synthetic construct
RADAAPTVSIFPPSSEQLTSGGASVVCFLNNFYPKDINVKWKIDGSERQNGVLNSWTDQDSKDSTYSMSSTLTLTKDEYERHNSYTCEATHKTSTSPIVKSFNRNEC

SEQ ID NO: 144 - protein, 449 aa, synthetic construct
EVQLVQSGAEVKKPGASVKVSCKASGYTFTSYYMHWVRQAPGQGLEWMGIINPGTGSTSHAQKFQGRVTMTRDTSTSTVYMELSSLRSEDTAVYYCARDGAFRHKYFDLWGRGTLVTVSSAKTTAPSVYPLAPVCGDTTGSSVTLGCLVKGYFPEPVTLTWNSGSLSSGVHTFPAVLQSDLYTLSSSVTVTSSTWPSQSITCNVAHPASSTKVDKKIEPRGPTIKPCPPCKCPAPNLLGGPSVFIFPPKIKDVLMISLSPIVTCVVVDVSEDDPDVQISWFVNNVEVHTAQTQTHREDYNSTLRVVSALPIQHQDWMSGKEFKCKVNNKDLPAPIERTISKPKGSVRAPQVYVLPPPEEEMTKKQVTLTCMVTDFMPEDIYVEWTNNGKTELNYKNTEPVLDSDGSYFMYSKLRVEKKNWVERNSYSCSVVHEGLHNHHTTKSFSRTPG

SEQ ID NO: 145 - protein, 214 aa, synthetic construct
EIVLTQSPATLSLSPGERATLSCRASQSVSSYLAWYQQKPGQAPRLLIYDASNRATGIPARFSGSGSGTDFTLTISSLEPEDFAVYYCQQYSAWPLTFGGGTKVEIKRADAAPTVSIFPPSSEQLTSGGASVVCFLNNFYPKDINVKWKIDGSERQNGVLNSWTDQDSKDSTYSMSSTLTLTKDEYERHNSYTCEATHKTSTSPIVKSFNRNEC

SEQ ID NO: 146 - protein, 447 aa, synthetic construct
EVQLVESGGGVVQPGRSLRLSCAASGFTFSSYTMHWVRQAPGKGLEWVTFISEDGNNKYYADSVKGRFTISRDNSKNTLYLQMNSLRAEDTAIYYCARTGWLGPFDYWGQGTLVTVSSAKTTAPSVYPLAPVCGDTTGSSVTLGCLVKGYFPEPVTLTWNSGSLSSGVHTFPAVLQSDLYTLSSSVTVTSSTWPSQSITCNVAHPASSTKVDKKIEPRGPTIKPCPPCKCPAPNLLGGPSVFIFPPKIKDVLMISLSPIVTCVVVDVSEDDPDVQISWFVNNVEVHTAQTQTHREDYNSTLRVVSALPIQHQDWMSGKEFKCKVNNKDLPAPIERTISKPKGSVRAPQVYVLPPPEEEMTKKQVTLTCMVTDFMPEDIYVEWTNNGKTELNYKNTEPVLDSDGSYFMYSKLRVEKKNWVERNSYSCSVVHEGLHNHHTTKSFSRTPG

SEQ ID NO: 147 - protein, 215 aa, synthetic construct
DIVLTQSPGTLSLSPGERATLSCRASQSVGSSYLAWYQQKPGQAPRLLIYGAFSRATGIPDRFSGSGSGTDFTLTISRLEPEDFAVYYCQQYGSSPWTFGQGTKVEIKRADAAPTVSIFPPSSEQLTSGGASVVCFLNNFYPKDINVKWKIDGSERQNGVLNSWTDQDSKDSTYSMSSTLTLTKDEYERHNSYTCEATHKTSTSPIVKSFNRNEC

SEQ ID NO: 148 - protein, 447 aa, synthetic construct
EVQLVESGGGVVQPGRSLRLSCAASGFTFSSYTMHWVRQAPGKGLEWVTFISEDGNNKYYADSVKGRFTISRDNSKNTLYLQMNSLRAEDTAIYYCARTGWLGPFDYWGQGTLVTVSSAKTTAPSVYPLAPVCGDTTGSSVTLGCLVKGYFPEPVTLTWNSGSLSSGVHTFPAVLQSDLYTLSSSVTVTSSTWPSQSITCNVAHPASSTKVDKKIEPRGPTIKPCPPCKCPAPNLLGGPSVFIFPPKIKDVLMISLSPIVTCVVVDVSEDDPDVQISWFVNNVEVHTAQTQTHREDYNSTLRVVSALPIQHQDWMSGKEFKCKVNNKDLPAPIERTISKPKGSVRAPQVYVLPPPEEEMTKKQVTLTCMVTDFMPEDIYVEWTNNGKTELNYKNTEPVLDSDGSYLMYSKLTVEKKNWVERNSYSCSVVHEGLHNHHTTKSFSRTPG

SEQ ID NO: 149 - protein, 449 aa, synthetic construct
EVQLVQSGAEVKKPGASVKVSCKASGYTFTSYYMHWVRQAPGQGLEWMGIINPGTGSTSHAQKFQGRVTMTRDTSTSTVYMELSSLRSEDTAVYYCARDGAFRHKYFDLWGRGTLVTVSSAKTTAPSVYPLAPVCGDTTGSSVTLGCLVKGYFPEPVTLTWNSGSLSSGVHTFPAVLQSDLYTLSSSVTVTSSTWPSQSITCNVAHPASSTKVDKKIEPRGPTIKPCPPCKCPAPNLLGGPSVFIFPPKIKDVLMISLSPIVTCVVVDVSEDDPDVQISWFVNNVEVHTAQTQTHREDYNSTLRVVSALPIQHQDWMSGKEFKCKVNNKDLPAPIERTISKPKGSVRAPQVYVLPPPEEEMTKKQVTLTCMVKDFMPEDIYVEWTNNGKTELNYKNTEPVLDSDGSYFMYSRLRVEKKNWVERNSYSCSVVHEGLHNRFTTKSFSRTPG

SEQ ID NO: 150 - protein, 215 aa, synthetic construct; identical to SEQ ID NO: 147

SEQ ID NO: 151 - protein, 214 aa, synthetic construct; identical to SEQ ID NO: 145

SEQ ID NO: 152 - protein, 447 aa, synthetic construct; identical to SEQ ID NO: 148

SEQ ID NO: 153 - protein, 449 aa, synthetic construct
EVQLVQSGAEVKKPGASVKVSCKASGYTFTSYYMHWVRQAPGQGLEWMGIINPMTGSASHAQKFQGRVTMTRDTSTSTVYMELSSLRSEDTAVYYCVRDAAARHKYFAFWGRGTLVTVSSAKTTAPSVYPLAPVCGDTTGSSVTLGCLVKGYFPEPVTLTWNSGSLSSGVHTFPAVLQSDLYTLSSSVTVTSSTWPSQSITCNVAHPASSTKVDKKIEPRGPTIKPCPPCKCPAPNLLGGPSVFIFPPKIKDVLMISLSPIVTCVVVDVSEDDPDVQISWFVNNVEVHTAQTQTHREDYNSTLRVVSALPIQHQDWMSGKEFKCKVNNKDLPAPIERTISKPKGSVRAPQVYVLPPPEEEMTKKQVTLTCMVKDFMPEDIYVEWTNNGKTELNYKNTEPVLDSDGSYFMYSRLRVEKKNWVERNSYSCSVVHEGLHNRFTTKSFSRTPG

SEQ ID NO: 154 - protein, 215 aa, synthetic construct; identical to SEQ ID NO: 147

SEQ ID NO: 155 - protein, 214 aa, synthetic construct; identical to SEQ ID NO: 145

SEQ ID NO: 156 - protein, 447 aa, synthetic construct
EVQLVESGGGVVQPGRSLRLSCAASGFTFSSYTMHWVRQAPGKGLEWVTFISEDGNNKYYADSVKGRFTISRDNSKNTLYLQMNSLRAEDTAIYYCARTGWLGPEDYWGQGTLVTVSSAKTTAPSVYPLAPVCGDTTGSSVTLGCLVKGYFPEPVTLTWNSGSLSSGVHTFPAVLQSDLYTLSSSVTVTSSTWPSQSITCNVAHPASSTKVDKKIEPRGPTIKPCPPCKCPAPNLLGGPSVFIFPPKIKDVLMISLSPIVTCVVVDVSEDDPDVQISWFVNNVEVHTAQTQTHREDYNSTLRVVSALPIQHQDWMSGKEFKCKVNNKDLPAPIERTISKPKGSVRAPQVYVLPPPEEEMTKKQVTLTCMVTDFMPEDIYVEWTNNGKTELNYKNTEPVLDSDGSYLMYSKLTVEKKNWVERNSYSCSVVHEGLHNHHTTKSFSRTPG

SEQ ID NO: 157 - protein, 449 aa, synthetic construct; identical to SEQ ID NO: 149

SEQ ID NO: 158 - protein, 215 aa, synthetic construct; identical to SEQ ID NO: 147

SEQ ID NO: 159 - protein, 214 aa, synthetic construct; identical to SEQ ID NO: 145

SEQ ID NO: 160 - protein, 454 aa, synthetic construct
QVQLQESGPGLVKPSETLSLTCTVSGFSLTSYGLSWIRQPPGKGLEWIGYIWYDGNTNFHSPLKSRVTISVDTSKNQFSLKLSSVTAADTAVYYCAKTEGHYYGSNYGYYALDYWGQGTLVTVSSASTKGPSVFPLAPSSKSTSGGTAALGCLVKDYFPEPVTVSWNSGALTSGVHTFPAVLQSSGLYSLSSVVTVPSSSLGTQTYICNVNHKPSNTKVDKKVEPKSCDKTHTCPPCPAPELLGGPSVFLFPPKPKDTLYITREPEVTCVVVDVSHEDPEVKFNWYVDGVEVHNAKTKPREEQYNATYRVVSVLTVLHQDWLNGKEYKCKVSNKALPAPIAATISKAKGQPREPQVYTLPPSRDELTKNQVSLTCLVKGFYPSDIAVEWESNGQPENNYKTTPPVLDSDGSFFLYSKLTVDKSRWQQGNVFSCSVMHEALHNHYTQKSLSLSPG

SEQ ID NO: 161 - protein, 214 aa, synthetic construct
DIQMTQSPSSLSASVGDRVTITCRASENIYSNLAWYQQKQGKAPKLLLYAATNLQDGVPSRFSGSGSGTDYTLTISSLQPEDFATYFCQHLWGTPYTFGQGTKLEIKRTVAAPSVFIFPPSDEQLKSGTASVVCLLNNFYPREAKVQWKVDNALQSGNSQESVTEQDSKDSTYSLSSTLTLSKADYEKHKVYACEVTHQGLSSPVTKSFNRGEC